European Patent Application EP 4 223 768 A1, published August 9, 2023. Title: Novel mutant bacteriorhodopsin-like channelrhodopsin ion channel. Applicant: Georg-August-Universität Göttingen Stiftung Öffentlichen Rechts, Universitätsmedizin OptoGenTech GmbH. The sequence listing filed with the application follows.

SEQUENCE LISTING (19 sequences)

SEQ ID NO: 1 - protein, 315 aa, Chlamydomonas reinhardtii
MDYGGALSAVGRELLFVTNPVVVNGSVLVPEDQCYCAGWIESRGTNGAQTASNVLQWLAAGFSILLLMFYAYQTWKSTCGWEEIYVCAIEMVKVILEFFFEFKNPSMLYLATGHRVQWLRYAEWLLTCPVILIHLSNLTGLSNDYSRRTMGLLVSDIGTIVWGATSAMATGYVKVIFFCLGLCYGANTFFHAAKAYIEGYHTVPKGRCRQVVTGMAWLFFVSWGMFPILFILGPEGFGVLSVYGSTVGHTIIDLMSKNCWGLLGHYLRVLIHEHILIHGDIRKTTKLNIGGTEIEVETLVEDEAEAGAVNKGTGK

SEQ ID NO: 2 - protein, 350 aa, Chlamydomonas noctigama
MAELISSATRSLFAAGGINPWPNPYHHEDMGCGGMTPTGECFSTEWWCDPSYGLSDAGYGYCFVEATGGYLVVGVEKKQAWLHSRGTPGEKIGAQVCQWIAFSIAIALLTFYGFSAWKATCGWEEVYVCCVEVLFVTLEIFKEFSSPATVYLSTGNHAYCLRYFEWLLSCPVILIKLSNLSGLKNDYSKRTMGLIVSCVGMIVFGMAAGLATDWLKWLLYIVSCIYGGYMYFQAAKCYVEANHSVPKGHCRMVVKLMAYAYFASWGSYPILWAVGPEGLLKLSPYANSIGHSICDIIAKEFWTFLAHHLRIKIHEHILIHGDIRKTTKMEIGGEEVEVEEFVEEEDEDTV

SEQ ID NO: 3 - protein, 300 aa, Artificial Sequence
  VChR1; channel rhodopsin 1 derived from Volvox carteri
MDYPVARSLIVRYPTDLGNGTVCMPRGQCYCEGWLRSRGTSIEKTIAITLQWVVFALSVACLGWYAYQAWRATCGWEEVYVALIEMMKSIIEAFHEFDSPATLWLSSGNGVVWMRYGEWLLTCPVLLIHLSNLTGLKDDYSKRTMGLLVSDVGCIVWGATSAMCTGWTKILFFLISLSYGMYTYFHAAKVYIEAFHTVPKGICRELVRVMAWTFFVAWGMFPVLFLLGTEGFGHISPYGSAIGHSILDLIAKNMWGVLGNYLRVKIHEHILLYGDIRKKQKITIAGQEMEVETLVAEEED

SEQ ID NO: 4 - protein, 350 aa, Artificial Sequence
  ReaChR; chimeric channelrhodopsin variant
MVSRRPWLLALALAVALAAGSAGASTGSDATVPVATQDGPDYVFHRAHERMLFQTSYTLENNGSVICIPNNGQCFCLAWLKSNGTNAEKLAANILQWVVFALSVACLGWYAYQAWRATCGWEEVYVALIEMMKSIIEAFHEFDSPATLWLSSGNGVVWMRYGEWLLTCPVILIHLSNLTGLKDDYSKRTMGLLVSDVGCIVWGATSAMCTGWTKILFFLISLSYGMYTYFHAAKVYIEAFHTVPKGLCRQLVRAMAWLFFVSWGMFPVLFLLGPEGFGHISPYGSAIGHSILDLIAKNMWGVLGNYLRVKIHEHILLYGDIRKKQKITIAGQEMEVETLVAEEEDKYESS

SEQ ID NO: 5 - protein, 309 aa, Artificial Sequence
  ChRmine; RICCR1; bacteriorhodopsin-like channelrhodopsin derived from Rhodomonas lens
MAHAPGTDQMFYVGTMDGWYLDTKLNSVAIGAHWSCFIVLTITTFYLGYESWTSRGPSKRTSFYAGYQEEQNLALFVNFFAMLSYFGKIVADTLGHNFGDVGPFIIGFGNYRYADYMLTCPMLVYDLLYQLRAPYRVSCSAIIFAILMSGVLAEFYAEGDPRLRNGAYAWYGFGCFWFIFAYSIVMSIVAKQYSRLAQLAQDTGAEHSLHVLKFAVFTFSMLWILFPLVWAICPRGFGWIDDNWTEVAHCVCDIVAKSCYGFALARFRKTYDEELFRLLEQLGHDEDEFQKLELDMRLSSNGERLRRLS

SEQ ID NO: 6 - protein, 309 aa, Artificial Sequence
  T218L mutant of ChRmine (RICCR1)
MAHAPGTDQMFYVGTMDGWYLDTKLNSVAIGAHWSCFIVLTITTFYLGYESWTSRGPSKRTSFYAGYQEEQNLALFVNFFAMLSYFGKIVADTLGHNFGDVGPFIIGFGNYRYADYMLTCPMLVYDLLYQLRAPYRVSCSAIIFAILMSGVLAEFYAEGDPRLRNGAYAWYGFGCFWFIFAYSIVMSIVAKQYSRLAQLAQDTGAEHSLHVLKFAVFLFSMLWILFPLVWAICPRGFGWIDDNWTEVAHCVCDIVAKSCYGFALARFRKTYDEELFRLLEQLGHDEDEFQKLELDMRLSSNGERLRRLS

SEQ ID NO: 7 - protein, 309 aa, Artificial Sequence
  S220A mutant of ChRmine (RICCR1)
MAHAPGTDQMFYVGTMDGWYLDTKLNSVAIGAHWSCFIVLTITTFYLGYESWTSRGPSKRTSFYAGYQEEQNLALFVNFFAMLSYFGKIVADTLGHNFGDVGPFIIGFGNYRYADYMLTCPMLVYDLLYQLRAPYRVSCSAIIFAILMSGVLAEFYAEGDPRLRNGAYAWYGFGCFWFIFAYSIVMSIVAKQYSRLAQLAQDTGAEHSLHVLKFAVFTFAMLWILFPLVWAICPRGFGWIDDNWTEVAHCVCDIVAKSCYGFALARFRKTYDEELFRLLEQLGHDEDEFQKLELDMRLSSNGERLRRLS

SEQ ID NO: 8 - protein, 309 aa, Artificial Sequence
  T218L+S220A mutant of ChRmine (RICCR1)
MAHAPGTDQMFYVGTMDGWYLDTKLNSVAIGAHWSCFIVLTITTFYLGYESWTSRGPSKRTSFYAGYQEEQNLALFVNFFAMLSYFGKIVADTLGHNFGDVGPFIIGFGNYRYADYMLTCPMLVYDLLYQLRAPYRVSCSAIIFAILMSGVLAEFYAEGDPRLRNGAYAWYGFGCFWFIFAYSIVMSIVAKQYSRLAQLAQDTGAEHSLHVLKFAVFLFAMLWILFPLVWAICPRGFGWIDDNWTEVAHCVCDIVAKSCYGFALARFRKTYDEELFRLLEQLGHDEDEFQKLELDMRLSSNGERLRRLS

SEQ ID NO: 9 - protein, 243 aa, Artificial Sequence
  7-transmembrane-helix motif of ChRmine (RICCR1)
SVAIGAHWSCFIVLTITTFYLGYESWTSRGPSKRTSFYAGYQEEQNLALFVNFFAMLSYFGKIVADTLGHNFGDVGPFIIGFGNYRYADYMLTCPMLVYDLLYQLRAPYRVSCSAIIFAILMSGVLAEFYAEGDPRLRNGAYAWYGFGCFWFIFAYSIVMSIVAKQYSRLAQLAQDTGAEHSLHVLKFAVFTFSMLWILFPLVWAICPRGFGWIDDNWTEVAHCVCDIVAKSCYGFALARFRK

SEQ ID NO: 10 - protein, 243 aa, Artificial Sequence
  T218L mutant of 7-transmembrane-helix motif of ChRmine (RICCR1)
SVAIGAHWSCFIVLTITTFYLGYESWTSRGPSKRTSFYAGYQEEQNLALFVNFFAMLSYFGKIVADTLGHNFGDVGPFIIGFGNYRYADYMLTCPMLVYDLLYQLRAPYRVSCSAIIFAILMSGVLAEFYAEGDPRLRNGAYAWYGFGCFWFIFAYSIVMSIVAKQYSRLAQLAQDTGAEHSLHVLKFAVFLFSMLWILFPLVWAICPRGFGWIDDNWTEVAHCVCDIVAKSCYGFALARFRK

SEQ ID NO: 11 - protein, 243 aa, Artificial Sequence
  S220A mutant of 7-transmembrane-helix motif of ChRmine (RICCR1)
SVAIGAHWSCFIVLTITTFYLGYESWTSRGPSKRTSFYAGYQEEQNLALFVNFFAMLSYFGKIVADTLGHNFGDVGPFIIGFGNYRYADYMLTCPMLVYDLLYQLRAPYRVSCSAIIFAILMSGVLAEFYAEGDPRLRNGAYAWYGFGCFWFIFAYSIVMSIVAKQYSRLAQLAQDTGAEHSLHVLKFAVFTFAMLWILFPLVWAICPRGFGWIDDNWTEVAHCVCDIVAKSCYGFALARFRK

SEQ ID NO: 12 - protein, 243 aa, Artificial Sequence
  T218L+S220A mutant of 7-transmembrane-helix motif of ChRmine (RICCR1)
SVAIGAHWSCFIVLTITTFYLGYESWTSRGPSKRTSFYAGYQEEQNLALFVNFFAMLSYFGKIVADTLGHNFGDVGPFIIGFGNYRYADYMLTCPMLVYDLLYQLRAPYRVSCSAIIFAILMSGVLAEFYAEGDPRLRNGAYAWYGFGCFWFIFAYSIVMSIVAKQYSRLAQLAQDTGAEHSLHVLKFAVFLFAMLWILFPLVWAICPRGFGWIDDNWTEVAHCVCDIVAKSCYGFALARFRK

SEQ ID NO: 13 - protein, 28 aa, Artificial Sequence
  variants of helix 6 motif of RICCR1
  VARIANT (14)..(14): in wild-type or wild-type like variant selected from T, S, Y, Q and N; in improved mutant selected from L, I, V, M, C, F, A, G, P and W
  VARIANT (16)..(16): in wild-type or wild-type like variant selected from S, T, Y, Q and N; in improved mutant selected from A, G, L, V, I, M, P, C and W
AEHSLHVLKFAVFXFXMLWILFPLVWAI

SEQ ID NO: 14 - DNA, 30 bp, Artificial Sequence
  forward primer humanized RICCR1 T218L
gttcgccgtgtttctgttctccatgctgtg

SEQ ID NO: 15 - DNA, 30 bp, Artificial Sequence
  reverse primer humanized RICCR1 T218L
cacagcatggagaacagaaacacggcgaac

SEQ ID NO: 16 - DNA, 28 bp, Artificial Sequence
  forward primer humanized RICCR1 S220A
gtgtttaccttcgccatgctgtggattc

SEQ ID NO: 17 - DNA, 28 bp, Artificial Sequence
  reverse primer humanized RICCR1 S220A
gaatccacagcatggcgaaggtaaacac

SEQ ID NO: 18 - DNA, 31 bp, Artificial Sequence
  forward primer humanized RICCR1 T218L+S220A
cgtgtttctgttcgccatgctgtggattctg

SEQ ID NO: 19 - DNA, 31 bp, Artificial Sequence
  reverse primer humanized RICCR1 T218L+S220A
cagaatccacagcatggcgaacagaaacacg